European Patent Specification EP 3 723 781 B1, published December 11, 2024. Title: PEPTIDES AND OTHER AGENTS FOR TREATING PAIN AND INCREASING PAIN SENSITIVITY. Applicant: The Research Foundation for the State University of New York. The sequence listing filed with the application follows.

SEQUENCE LISTING (113 sequences)

SEQ ID NO: 1 - protein, 15 aa, Artificial Sequence
  Synthetic peptide
STAACPPSYDRVTKP

SEQ ID NO: 2 - protein, 15 aa, Artificial Sequence
  Synthetic peptide
PSTTSPPSYDSVTKP

SEQ ID NO: 3 - protein, 15 aa, Artificial Sequence
  Synthetic peptide
SSTTSPPSYDSVTKP

SEQ ID NO: 4 - protein, 15 aa, Artificial Sequence
  Synthetic peptide
SSTSFPPSYDSVTRA

SEQ ID NO: 5 - protein, 15 aa, Artificial Sequence
  Synthetic peptide
PSTASLPSYDSVTKP

SEQ ID NO: 6 - protein, 15 aa, Artificial Sequence
  Synthetic peptide
SSTTSPPSYDSVTKP

SEQ ID NO: 7 - protein, 15 aa, Artificial Sequence
  Synthetic peptide
SATSFPPSYESVTRG

SEQ ID NO: 8 - protein, 15 aa, Artificial Sequence
  Synthetic peptide
  MISC_FEATURE (13)..(13): The peptide of this residue is phosphorylated.
STAACPPSYDRVTKP

SEQ ID NO: 9 - protein, 15 aa, Artificial Sequence
  Synthetic peptide
  MISC_FEATURE (13)..(13): The peptide of this residue is phosphorylated.
PSTTSPPSYDSVTKP

SEQ ID NO: 10 - protein, 15 aa, Artificial Sequence
  Synthetic peptide
  MISC_FEATURE (13)..(13): The peptide of this residue is phosphorylated.
SSTTSPPSYDSVTKP

SEQ ID NO: 11 - protein, 15 aa, Artificial Sequence
  Synthetic peptide
  MISC_FEATURE (13)..(13): The peptide of this residue is phosphorylated.
SSTSFPPSYDSVTRA

SEQ ID NO: 12 - protein, 15 aa, Artificial Sequence
  Synthetic peptide
  MISC_FEATURE (13)..(13): The peptide of this residue is phosphorylated.
PSTASLPSYDSVTKP

SEQ ID NO: 13 - protein, 15 aa, Artificial Sequence
  Synthetic peptide
  MISC_FEATURE (13)..(13): The peptide of this residue is phosphorylated.
SSTTSPPSYDSVTKP

SEQ ID NO: 14 - protein, 15 aa, Artificial Sequence
  Synthetic peptide
  MISC_FEATURE (13)..(13): The peptide of this residue is phosphorylated.
SATSFPPSYESVTRG

SEQ ID NO: 15 - protein, 15 aa, Artificial Sequence
  Synthetic peptide
STAACPPSYDRVAKP

SEQ ID NO: 16 - protein, 15 aa, Artificial Sequence
  Synthetic peptide
PSTTSPPSYDSVAKP

SEQ ID NO: 17 - protein, 15 aa, Artificial Sequence
  Synthetic peptide
SSTTSPPSYDSVAKP

SEQ ID NO: 18 - protein, 15 aa, Artificial Sequence
  Synthetic peptide
SSTSFPPSYDSVARA

SEQ ID NO: 19 - protein, 15 aa, Artificial Sequence
  Synthetic peptide
PSTASLPSYDSVAKP

SEQ ID NO: 20 - protein, 15 aa, Artificial Sequence
  Synthetic peptide
SSTTSPPSYDSVAKP

SEQ ID NO: 21 - protein, 15 aa, Artificial Sequence
  Synthetic peptide
SATSFPPSYESVARG

SEQ ID NO: 22 - protein, 15 aa, Artificial Sequence
  Synthetic peptide
STAACPPSYDRVEKP

SEQ ID NO: 23 - protein, 15 aa, Artificial Sequence
  Synthetic peptide
PSTTSPPSYDSVEKP

SEQ ID NO: 24 - protein, 15 aa, Artificial Sequence
  Synthetic peptide
SSTTSPPSYDSVEKP

SEQ ID NO: 25 - protein, 15 aa, Artificial Sequence
  Synthetic peptide
SSTSFPPSYDSVERA

SEQ ID NO: 26 - protein, 15 aa, Artificial Sequence
  Synthetic peptide
PSTASLPSYDSVEKP

SEQ ID NO: 27 - protein, 15 aa, Artificial Sequence
  Synthetic peptide
SSTTSPPSYDSVEKP

SEQ ID NO: 28 - protein, 15 aa, Artificial Sequence
  Synthetic peptide
SATSFPPSYESVERG

SEQ ID NO: 29 - protein, 15 aa, Artificial Sequence
  Synthetic peptide
STAACPPSYDRVDKP

SEQ ID NO: 30 - protein, 15 aa, Artificial Sequence
  Synthetic peptide
PSTTSPPSYDSVDKP

SEQ ID NO: 31 - protein, 15 aa, Artificial Sequence
  Synthetic peptide
SSTTSPPSYDSVDKP

SEQ ID NO: 32 - protein, 15 aa, Artificial Sequence
  Synthetic peptide
SSTSFPPSYDSVDRA

SEQ ID NO: 33 - protein, 15 aa, Artificial Sequence
  Synthetic peptide
PSTASLPSYDSVDKP

SEQ ID NO: 34 - protein, 15 aa, Artificial Sequence
  Synthetic peptide
SSTTSPPSYDSVDKP

SEQ ID NO: 35 - protein, 15 aa, Artificial Sequence
  Synthetic peptide
SATSFPPSYESVDRG

SEQ ID NO: 36 - protein, 15 aa, Artificial Sequence
  Synthetic peptide
  MISC_FEATURE (1)..(1): The peptide of this residue is myristoylated.
STAACPPSYDRVTKP

SEQ ID NO: 37 - protein, 15 aa, Artificial Sequence
  Synthetic peptide
  MISC_FEATURE (1)..(1): The residue at this position is phosphorylated.
PSTTSPPSYDSVTKP

SEQ ID NO: 38 - protein, 15 aa, Artificial Sequence
  Synthetic peptide
  MISC_FEATURE (1)..(1): The peptide of this residue is myristoylated.
SSTTSPPSYDSVTKP

SEQ ID NO: 39 - protein, 15 aa, Artificial Sequence
  Synthetic peptide
SSTSFPPSYDSVTRA

SEQ ID NO: 40 - protein, 15 aa, Artificial Sequence
  Synthetic peptide
  MISC_FEATURE (1)..(1): The peptide of this residue is myristoylated.
SSTASLPSYDSVTKP

SEQ ID NO: 41 - protein, 15 aa, Artificial Sequence
  Synthetic peptide
  MISC_FEATURE (1)..(1): The peptide of this residue is myristoylated.
SSTISPPSYDSVTKP

SEQ ID NO: 42 - protein, 15 aa, Artificial Sequence
  Synthetic peptide
  MISC_FEATURE (1)..(1): The peptide of this residue is myristoylated.
SATSFPPSYDSVTRG

SEQ ID NO: 43 - protein, 15 aa, Artificial Sequence
  Synthetic peptide
  MISC_FEATURE (1)..(1): The peptide of this residue is myristoylated.
  MISC_FEATURE (13)..(13): The peptide of this residue is phosphorylated.
STAACPPSYDRVTKP

SEQ ID NO: 44 - protein, 15 aa, Artificial Sequence
  Synthetic peptide
  MISC_FEATURE (1)..(1): The residue at this position is phosphorylated.
  MISC_FEATURE (13)..(13): The peptide of this residue is phosphorylated.
PSTTSPPSYDSVTKP

SEQ ID NO: 45 - protein, 15 aa, Artificial Sequence
  Synthetic peptide
  MISC_FEATURE (1)..(1): The peptide of this residue is myristoylated.
  MISC_FEATURE (13)..(13): The peptide of this residue is phosphorylated.
SSTTSPPSYDSVTKP

SEQ ID NO: 46 - protein, 15 aa, Artificial Sequence
  Synthetic peptide
  MISC_FEATURE (1)..(1): The peptide of this residue is myristoylated.
  MISC_FEATURE (13)..(13): The peptide of this residue is phosphorylated.
SSTSFPPSYDSVTRA

SEQ ID NO: 47 - protein, 15 aa, Artificial Sequence
  Synthetic peptide
  MISC_FEATURE (1)..(1): The peptide of this residue is myristoylated.
  MISC_FEATURE (13)..(13): The peptide of this residue is phosphorylated.
SSTASLPSYDSVTKP

SEQ ID NO: 48 - protein, 15 aa, Artificial Sequence
  Synthetic peptide
  MISC_FEATURE (1)..(1): The peptide of this residue is myristoylated.
  MISC_FEATURE (13)..(13): The peptide of this residue is phosphorylated.
SSTISPPSYDSVTKP

SEQ ID NO: 49 - protein, 15 aa, Artificial Sequence
  Synthetic peptide
  MISC_FEATURE (1)..(1): The peptide of this residue is myristoylated.
  MISC_FEATURE (13)..(13): The peptide of this residue is phosphorylated.
SATSFPPSYDSVTRG

SEQ ID NO: 50 - protein, 15 aa, Artificial Sequence
  Synthetic peptide
  MISC_FEATURE (1)..(1): The peptide of this residue is myristoylated.
STAACPPSYDRVAKP

SEQ ID NO: 51 - protein, 15 aa, Artificial Sequence
  Synthetic peptide
  MISC_FEATURE (1)..(1): The residue at this position is phosphorylated.
PSTTSPPSYDSVAKP

SEQ ID NO: 52 - protein, 15 aa, Artificial Sequence
  Synthetic peptide
  MISC_FEATURE (1)..(1): The peptide of this residue is myristoylated.
SSTTSPPSYDSVAKP

SEQ ID NO: 53 - protein, 15 aa, Artificial Sequence
  Synthetic peptide
  MISC_FEATURE (1)..(1): The peptide of this residue is myristoylated.
SSTSFPPSYDSVARA

SEQ ID NO: 54 - protein, 15 aa, Artificial Sequence
  Synthetic peptide
  MISC_FEATURE (1)..(1): The peptide of this residue is myristoylated.
SSTASLPSYDSVAKP

SEQ ID NO: 55 - protein, 15 aa, Artificial Sequence
  Synthetic peptide
  MISC_FEATURE (1)..(1): The peptide of this residue is myristoylated.
SSTISPPSYDSVAKP

SEQ ID NO: 56 - protein, 15 aa, Artificial Sequence
  Synthetic peptide
  MISC_FEATURE (1)..(1): The peptide of this residue is myristoylated.
SATSFPPSYDSVARG

SEQ ID NO: 57 - protein, 15 aa, Artificial Sequence
  Synthetic peptide
  MISC_FEATURE (1)..(1): The peptide of this residue is myristoylated.
STAACPPSYDRVEKP

SEQ ID NO: 58 - protein, 15 aa, Artificial Sequence
  Synthetic peptide
  MISC_FEATURE (1)..(1): The residue at this position is phosphorylated.
PSTTSPPSYDSVEKP

SEQ ID NO: 59 - protein, 15 aa, Artificial Sequence
  Synthetic peptide
  MISC_FEATURE (1)..(1): The peptide of this residue is myristoylated.
SSTTSPPSYDSVEKP

SEQ ID NO: 60 - protein, 15 aa, Artificial Sequence
  Synthetic peptide
  MISC_FEATURE (1)..(1): The peptide of this residue is myristoylated.
SSTSFPPSYDSVERA

SEQ ID NO: 61 - protein, 15 aa, Artificial Sequence
  Synthetic peptide
  MISC_FEATURE (1)..(1): The peptide of this residue is myristoylated.
SSTASLPSYDSVEKP

SEQ ID NO: 62 - protein, 15 aa, Artificial Sequence
  Synthetic peptide
  MISC_FEATURE (1)..(1): The peptide of this residue is myristoylated.
SSTISPPSYDSVEKP

SEQ ID NO: 63 - protein, 15 aa, Artificial Sequence
  Synthetic peptide
  MISC_FEATURE (1)..(1): The peptide of this residue is myristoylated.
SATSFPPSYDSVERG

SEQ ID NO: 64 - protein, 15 aa, Artificial Sequence
  Synthetic peptide
  MISC_FEATURE (1)..(1): The peptide of this residue is myristoylated.
STAACPPSYDRVDKP

SEQ ID NO: 65 - protein, 15 aa, Artificial Sequence
  Synthetic peptide
  MISC_FEATURE (1)..(1): The residue at this position is phosphorylated.
PSTTSPPSYDSVDKP

SEQ ID NO: 66 - protein, 15 aa, Artificial Sequence
  Synthetic peptide
  MISC_FEATURE (1)..(1): The peptide of this residue is myristoylated.
SSTTSPPSYDSVDKP

SEQ ID NO: 67 - protein, 15 aa, Artificial Sequence
  Synthetic peptide
  MISC_FEATURE (1)..(1): The peptide of this residue is myristoylated.
SSTSFPPSYDSVDRA

SEQ ID NO: 68 - protein, 15 aa, Artificial Sequence
  Synthetic peptide
  MISC_FEATURE (1)..(1): The peptide of this residue is myristoylated.
SSTASLPSYDSVDKP

SEQ ID NO: 69 - protein, 15 aa, Artificial Sequence
  Synthetic peptide
  MISC_FEATURE (1)..(1): The peptide of this residue is myristoylated.
SSTISPPSYDSVDKP

SEQ ID NO: 70 - protein, 15 aa, Artificial Sequence
  Synthetic peptide
  MISC_FEATURE (1)..(1): The peptide of this residue is myristoylated.
SATSFPPSYDSVDRG

SEQ ID NO: 71 - protein, 4 aa, Artificial Sequence
  Synthetic peptide
  X (1)..(1): P or L
  X (3)..(3): Any amino acid residue
XPXY

SEQ ID NO: 72 - protein, 4 aa, Artificial Sequence
  Synthetic peptide
TAAC

SEQ ID NO: 73 - protein, 4 aa, Artificial Sequence
  Synthetic peptide
PPSY

SEQ ID NO: 74 - protein, 6 aa, Artificial Sequence
  Synthetic peptide
DRVTKP

SEQ ID NO: 75 - protein, 15 aa, Artificial Sequence
  Synthetic Peptide
  X1 (1)..(1): X1 is selected from the group consisting of S, P, and A.
  X1 (1)..(1): The residue at this position is acylated at a nucleophilic atom of the amino acid residue.
  X2 (2)..(2): X2 is selected from the group consisting of T, S, and A.
  X2 (2)..(2): The residue at this position is acylated at a nucleophilic atom of the amino acid residue.
  X3 (3)..(3): X3 is selected from the group consisting of A and T.
  X3 (3)..(3): The residue at this position is acylated at a nucleophilic atom of the amino acid residue.
  X4 (4)..(4): X4 is selected from the group consisting of A, T, I, and S.
  X4 (4)..(4): The residue at this position is acylated at a nucleophilic atom of the amino acid residue.
  X5 (5)..(5): X5 is selected from the group consisting of C, S, and F
  X6 (6)..(6): X6 is selected from the group consisting of P and L
  X7 (8)..(8): X7 is any amino acid residue.
  X8 (10)..(10): X8 is selected from the group consisting of E, D and Y.
  X9 (11)..(11): X9 is selected from the group consisting of S and R.
  X10 (13)..(13): X10 is selected from the group consisting of T, A, E, and D, and T is phosphorylated.
  X10 (13)..(13): The residue at this position is acylated at a nucleophilic atom of the amino acid residue.
  X11 (14)..(14): X11 is selected from the group consisting of K and R.
  X11 (14)..(14): The residue at this position is acylated at a nucleophilic atom of the amino acid residue.
  X12 (15)..(15): X12 is selected from the group consisting of P, A, and G.
XXXXXXPXYXXVXXX

SEQ ID NO: 76 - protein, 4 aa, Artificial Sequence
  Synthetic peptide
  X3 (3)..(3): X is any amino acid residue.
PPXY

SEQ ID NO: 77 - protein, 15 aa, Artificial Sequence
  Synthetic peptide
  MISC_FEATURE (1)..(1): The peptide of this residue is myristoylated.
  MISC_FEATURE (13)..(13): The peptide of this residue is phosphorylated.
SATSFPPSYDSVTRG

SEQ ID NO: 78 - protein, 4 aa, Artificial Sequence
  Synthetic peptide
PPRY

SEQ ID NO: 79 - protein, 10 aa, Artificial Sequence
  Synthetic peptide
NPETRDETQL

SEQ ID NO: 80 - protein, 10 aa, Artificial Sequence
  Synthetic peptide
QPNTRLDETE

SEQ ID NO: 81 - protein, 14 aa, Artificial Sequence
  Synthetic peptide
SDRPVTSYSFSAPG

SEQ ID NO: 82 - DNA, 30 bp, Artificial Sequence
  Primer
gtcttcgagggggccgagaatataacatgg

SEQ ID NO: 83 - DNA, 22 bp, Artificial Sequence
  Primer
ggtggaggggccgttcctgtcg

SEQ ID NO: 84 - DNA, 21 bp, Artificial Sequence
  Primer
cccaaagggcagcaggagctg

SEQ ID NO: 85 - DNA, 22 bp, Artificial Sequence
  Primer
cggcgagtgcagccttctgtga

SEQ ID NO: 86 - DNA, 24 bp, Artificial Sequence
  Primer
ctgccacaagtccaaaagtgtgaa

SEQ ID NO: 87 - DNA, 22 bp, Artificial Sequence
  Primer
agtcatcgggctcgtccagatc

SEQ ID NO: 88 - RNA, 21 nt, Artificial Sequence
  siRNA
ggaaagacagccagaauaguu

SEQ ID NO: 89 - RNA, 21 nt, Artificial Sequence
  siRNA
gcccaagcuccagaucaaacu

SEQ ID NO: 90 - RNA, 21 nt, Artificial Sequence
  siRNA
guggaugggacgccaguaauu

SEQ ID NO: 91 - RNA, 21 nt, Artificial Sequence
  siRNA
gaagcauucucgagcuauaga

SEQ ID NO: 92 - RNA, 21 nt, Artificial Sequence
  siRNA
guuuccccuauucaccagugu

SEQ ID NO: 93 - RNA, 21 nt, Artificial Sequence
  siRNA
gccucucgcaccaugugauua

SEQ ID NO: 94 - RNA, 21 nt, Artificial Sequence
  siRNA
gaccaagagcgaaggaauguu

SEQ ID NO: 95 - RNA, 21 nt, Artificial Sequence
  siRNA
guuccucagauccaauuguua

SEQ ID NO: 96 - RNA, 21 nt, Artificial Sequence
  siRNA
gaccaucugagcccacuacua

SEQ ID NO: 97 - RNA, 21 nt, Artificial Sequence
  siRNA
ggaaacaugugacuauaccuu

SEQ ID NO: 98 - RNA, 21 nt, Artificial Sequence
  siRNA
gaucuuuacauagcuuagugu

SEQ ID NO: 99 - protein, 4 aa, Artificial Sequence
  Synthetic peptide
ETQL

SEQ ID NO: 100 - protein, 48 aa, Xenopus
RLELNDIVYLIRSDPLAHVANESHSRKSSNSYKTDPVGNPETRDETQL

SEQ ID NO: 101 - protein, 47 aa, Gallus gallus
RLELNDIVYLIRSDPLAHVANDGHSRKSSCSNKLGPCNPETRDETQL

SEQ ID NO: 102 - protein, 47 aa, Rattus norvegicus
RLEPNDIVYLIRSDPLAHVTSSSQSRKSSCSNKLSSCNPETRDETQL

SEQ ID NO: 103 - protein, 47 aa, Homo sapiens
RLEPSDIVYLIRSDPLAHVASSSQSRKSSCSHKLSSCNPETRDETQL

SEQ ID NO: 104 - protein, 44 aa, Rattus norvegicus
RLELNDVVYLIRPDPLSYLPNSEPSRKNSICNAAVQDSREETQL

SEQ ID NO: 105 - protein, 15 aa, Rattus norvegicus
STAACPPSYDRVTKP

SEQ ID NO: 106 - protein, 15 aa, Rattus norvegicus
PSTTSPPSYDSVTKP

SEQ ID NO: 107 - protein, 15 aa, Rattus norvegicus
SSTTSPPSYDSVTKP

SEQ ID NO: 108 - protein, 15 aa, Rattus norvegicus
SSTSFPPSYDSVTRA

SEQ ID NO: 109 - protein, 15 aa, Rattus norvegicus
ASTISPPSYDSVTKP

SEQ ID NO: 110 - protein, 15 aa, Rattus norvegicus
SATSFPPSYDSVTRG

SEQ ID NO: 111 - protein, 15 aa, Rattus norvegicus
PSTASLPSYDSVTKP

SEQ ID NO: 112 - protein, 4 aa, Xenopus
ETQL

SEQ ID NO: 113 - protein, 10 aa, Artificial Sequence
  Synthetic peptide
  MISC_FEATURE (1)..(1): The peptide of this residue is myristoylated.
QPNTRLDETE